European Patent Application EP 4 450 628 A1, published October 23, 2024. Title: NUCELEIC ACID EXPRESSION PLATFORM INCREASING EXPRESSION EFFICIENCY. Applicant: SML Biopharm Co., Ltd. Application KR. The sequence listing filed with the application follows.

SEQUENCE LISTING (19 sequences)

SEQ ID NO: 1 - DNA, 57 bp, Homo sapiens
  source 1..57: mol_type = genomic DNA
agcaaggctcagcctcaagattcacagcatctcagacacagcctaggccgcaccagg

SEQ ID NO: 2 - DNA, 41 bp, Homo sapiens
  source 1..41: mol_type = genomic DNA
ctagcttttctcttctgtcaaccccacacgcctttggcaca

SEQ ID NO: 3 - DNA, 199 bp, Homo sapiens
  source 1..199: mol_type = genomic DNA
gcagttcggcggtcccgcgggtctgtctcttgcttcaacagtgtttggacggaacagatccggggactctcttccagcctccgaccgccctccgatttcctctccgcttgcaacctccgggaccatcttctcggccatctcctgcttctgggacctgccagcaccgtttttgtggttagctccttcttgccaaccaacc

SEQ ID NO: 4 - DNA, 137 bp, Homo sapiens
  source 1..137: mol_type = genomic DNA
attcccagcctcacatcactcacaccttgcatttcacccctgcatcccagtcgccctgcagcctcacacagatcctgcacacacccagacagctggcgctcacacattcaccgttggcctgcctctgttcaccctcc

SEQ ID NO: 5 - DNA, 51 bp, Homo sapiens
  source 1..51: mol_type = genomic DNA
gactctgggaggcgtttgggcccagagaagtggatccgccgcttgcgccgc

SEQ ID NO: 6 - DNA, 35 bp, Homo sapiens
  source 1..35: mol_type = genomic DNA
cctttccggcggtgacgacctacgcacacgagaac

SEQ ID NO: 7 - DNA, 42 bp, Homo sapiens
  source 1..42: mol_type = genomic DNA
acatatccactcctgctctccctcctgcaggtgaccccagcc

SEQ ID NO: 8 - DNA, 217 bp, Homo sapiens
  source 1..217: mol_type = genomic DNA
ggatgccgccccggacagtggcacctgggaagcctgggagtgtttgtcccatcggtagcttgaaataaacgctcccctcagacacccgctgggttctctgatgttattatggttgagatgcagctggtctctcctggttaattgacttcttattaccaacaagttacttgaaagagtgtcaccaataatcattaaagtacggcaggctgaaccttca

SEQ ID NO: 9 - DNA, 186 bp, Homo sapiens
  source 1..186: mol_type = genomic DNA
gatcacatttaaaagcatctcagcctaccatgagaataagagaaagaaaatgaagatcaaaagcttattcatctgtttttctttttcgttggtgtaaagccaacaccctgtctaaaaaacataaatttctttaatcattttgcctcttttctctgtgcttcaattaataaaaaatggaaagaatcg

SEQ ID NO: 10 - DNA, 144 bp, Homo sapiens
  source 1..144: mol_type = genomic DNA
gagccttctgagcccagcgacttctgaagggccccttgcaaagtaatagggcttctgcctaagcctctccctccagccaataggcagctttcttaactatcctaacaagccttggaccaaatggaaataaagctttttgatgca

SEQ ID NO: 11 - DNA, 248 bp, Homo sapiens
  source 1..248: mol_type = genomic DNA
gctatgaccgtgcagagggagcccggagtccgagtcaagcattgtgaattattacctaacctggggaaccgaggaccagaaggaaggaccaggcttccagctcctctgcaccagacctgaccagccaggacagggcctggggtgtgtgtgagtgtgagtgtgagcgagagggtgagtgtggtcagagtaaagctgctccacccccagattgcaatgctaccaataaagccgcctggtgtttacaacta

SEQ ID NO: 12 - DNA, 400 bp, Homo sapiens
  source 1..400: mol_type = genomic DNA
tggctgcagcccctgcctgtgtgtctggtgttgaggggacgaagggacccctgcccctgtctgccagcagaggcagtagggcacagagggaagaggagggtggggccctggatgactttccagcctcttcaactgacttgctcccctctccttttcttctctttagagacccagcccagggccctcccacccttgcccagacctggtgggcccttcagagggaggggtggacctgtttctctttcactttcatttgctggtgtgagccatggggtgtgtatttgtatgtggggagtaggtgtttgaggttcccgttctttcccttcccaagtctctgggggtggaaaggaggaagagatactagttaaagattttaaaaatgtaaataaaatatacttcc

SEQ ID NO: 13 - DNA, 54 bp, Homo sapiens
  source 1..54: mol_type = genomic DNA
aagcactctgagtcaagatgagtgggaaaccatctcaataaacacattttggat

SEQ ID NO: 14 - DNA, 126 bp, Homo sapiens
  source 1..126: mol_type = genomic DNA
gcttcctagatagaaaccaaagcagtgcaagattcagttcaaggtcctgaaaaaagaaaaacattttactctgtgtaccttgtgtctttctaaatttctctctccaaaataaagttcaagcattaa

SEQ ID NO: 15 - DNA, 936 bp, synthetic construct
  source 1..936: mol_type = other DNA
atgacttcgaaagtttatgatccagaacaaaggaaacggatgataactggtccgcagtggtgggccagatgtaaacaaatgaatgttcttgattcatttattaattattatgattcagaaaaacatgcagaaaatgctgttatttttttacatggtaacgcggcctcttcttatttatggcgacatgttgtgccacatattgagccagtagcgcggtgtattataccagaccttattggtatgggcaaatcaggcaaatctggtaatggttcttataggttacttgatcattacaaatatcttactgcatggtttgaacttcttaatttaccaaagaagatcatttttgtcggccatgattggggtgcttgtttggcatttcattatagccatgagcatcaagataagatcaaagcaatagttcacgctgaaagtgtagtagatgtgattgaatcatgggatgaatggcctgatattgaagaagatattgcgttgatcaaatctgaagaaggagaaaaaatggttttggagaataacttcttcgtggaaaccatgttgccatcaaaaatcatgagaaagttagaaccagaagaatttgcagcatatcttgaaccattcaaagagaaaggtgaagttcgtcgtccaacattatcatggcctcgtgaaatcccgttagtaaaaggtggtaaacctgacgttgtacaaattgttaggaattataatgcttatctacgtgcaagtgatgatttaccaaaaatgtttattgaatcggacccaggattcttttccaatgctattgttgaaggtgccaagaagtttcctaatactgaatttgtcaaagtaaaaggtcttcatttttcgcaagaagatgcacctgatgaaatgggaaaatatatcaaatcgttcgttgagcgagttctcaaaaatgaacaataa

SEQ ID NO: 16 - DNA, 19 bp, Bacteriophage T7
  source 1..19: mol_type = genomic DNA
taatacgactcactatagg

SEQ ID NO: 17 - DNA, 110 bp, synthetic construct
  source 1..110: mol_type = other DNA
aaaaaaaaaaaaaaaaaaaaaaaaaaaaaaaaaaaaaaaaaaaaaaaaaagatcatcagtaaaaaaaaaaaaaaaaaaaaaaaaaaaaaaaaaaaaaaaaaaaaaaaaaa

SEQ ID NO: 18 - DNA, 2223 bp, synthetic construct
  source 1..2223: mol_type = other DNA
gtggcacttttcggggaaatgtgcgcggaacccctatttgtttatttttctaaatacattcaaatatgtatccgctcatgagacaataaccctgataaatgcttcaataatattgaaaaaggaagagtatgagtattcaacatttccgtgtcgcccttattcccttttttgcggcattttgccttcctgtttttgctcacccagaaacgctggtgaaagtaaaagatgctgaagatcagttgggtgcacgagtgggttacatcgaactggatctcaacagcggtaagatccttgagagttttcgccccgaagaacgttttccaatgatgagcacttttaaagttctgctatgtggcgcggtattatcccgtattgacgccgggcaagagcaactcggtcgccgcatacactattctcagaatgacttggttgagtactcaccagtcacagaaaagcatcttacggatggcatgacagtaagagaattatgcagtgctgccataaccatgagtgataacactgcggccaacttacttctgacaacgatcggaggaccgaaggagctaaccgcttttttgcacaacatgggggatcatgtaactcgccttgatcgttgggaaccggagctgaatgaagccataccaaacgacgagcgtgacaccacgatgcctgtagcaatggcaacaacgttgcgcaaactattaactggcgaactacttactctagcttcccggcaacaattaatagactggatggaggcggataaagttgcaggaccacttctgcgctcggcccttccggctggctggtttattgctgataaatctggagccggtgagcgtggatctcgcggtatcattgcagcactggggccagatggtaagccctcccgtatcgtagttatctacacgacggggagtcaggcaactatggatgaacgaaatagacagatcgctgagataggtgcctcactgattaagcattggtaactgtcagaccaagtttactcatatatactttagattgatttaaaacttcatttttaatttaaaaggatctaggtgaagatcctttttgataatctcatgaccaaaatcccttaacgtgagttttcgttccactgagcgtcagaccccgtagaaaagatcaaaggatcttcttgagatcctttttttctgcgcgtaatctgctgcttgcaaacaaaaaaaccaccgctaccagcggtggtttgtttgccggatcaagagctaccaactctttttccgaaggtaactggcttcagcagagcgcagataccaaatactgtccttctagtgtagccgtagttaggccaccacttcaagaactctgtagcaccgcctacatacctcgctctgctaatcctgttaccagtggctgctgccagtggcgataagtcgtgtcttaccgggttggactcaagacgatagttaccggataaggcgcagcggtcgggctgaacggggggttcgtgcacacagcccagcttggagcgaacgacctacaccgaactgagatacctacagcgtgagctatgagaaagcgccacgcttcccgaagggagaaaggcggacaggtatccggtaagcggcagggtcggaacaggagagcgcacgagggagcttccagggggaaacgcctggtatctttatagtcctgtcgggtttcgccacctctgacttgagcgtcgatttttgtgatgctcgtcaggggggcggagcctatggaaaaacgccagcaacgcggcctttttacggttcctggccttttgctggccttttgctcacatgttctttcctgcgttatcccctgattctgtggataaccgtattaccgcctttgagtgagctgataccgctcgccgcagccgaacgaccgagcgcagcgagtcagtgagcgaggaagcggaagagcgcccaatacgcaaaccgcctctccccgcgcgttggccgattcattaatgcagctggcacgacaggtttcccgactggaaagcgggcagtgagcgcaacgcaattaatgtgagttagctcactcattaggcaccccaggctttacactttatgcttccggctcgtatgttgtgtggaattgtgagcggataacaatttcacacaggaaacagctatgaccatgattacgccaagcgcgcaattaaccctcactaaagggaacaaaagctggagcttgcaagcttcacgtgat

SEQ ID NO: 19 - DNA, 15 bp, synthetic construct
  source 1..15: mol_type = other DNA
gaagagcgcggccgc